European Patent Specification EP 3 149 026 B1, published March 5, 2025. Title: SITE-SELECTIVE MODIFICATION OF POLYSACCHARIDES AND APPLICATIONS THEREOF. Applicant: B.G. Negev Technologies and Applications Ltd. The sequence listing filed with the application follows.

SEQUENCE LISTING (6 sequences)

SEQ ID NO: 1 - protein, 8 aa, Artificial Sequence
  synthetic
GGGGRGDY

SEQ ID NO: 2 - protein, 11 aa, Artificial Sequence
  synthetic
GGGKGGGRGDY

SEQ ID NO: 3 - protein, 13 aa, Artificial Sequence
  synthetic
GGGGRGDYKFITC

SEQ ID NO: 4 - protein, 14 aa, Artificial Sequence
  synthetic
GGGGSPPRRARVTY

SEQ ID NO: 5 - protein, 14 aa, Artificial Sequence
  synthetic
GGGGSPPLLALVTY

SEQ ID NO: 6 - protein, 15 aa, Artificial Sequence
  synthetic
GGGGSPPRRARVTYK